European Patent Specification EP 4 281 099 B1, published October 1, 2025. Title: COMPOSITIONS COMPRISING PEDF-DERIVED SHORT PEPTIDES (PDSP) AND USES THEREOF. Applicant: BRIM Biotechnology, Inc. The sequence listing filed with the application follows.

SEQUENCE LISTING (9 sequences)

SEQ ID NO: 1 - protein, 39 aa, Artificial Sequence
  Synthetic
LSVATALSALSLGAEQRTESIIHRALYYDLISSPDIHGT

SEQ ID NO: 2 - protein, 34 aa, Artificial Sequence
  Synthetic
ALSALSLGAEQRTESIIHRALYYDLISSPDIHGT

SEQ ID NO: 3 - protein, 29 aa, Artificial Sequence
  Synthetic
SLGAEQRTESIIHRALYYDLISSPDIHGT

SEQ ID NO: 4 - protein, 25 aa, Artificial Sequence
  Synthetic
EQRTESIIHRALYYDLISSPDIHGT

SEQ ID NO: 5 - protein, 24 aa, Artificial Sequence
  Synthetic
SLGAEQRTESIIHRALYYDLISSP

SEQ ID NO: 6 - protein, 20 aa, Artificial Sequence
  Synthetic
SLGAEQRTESIIHRALYYDL

SEQ ID NO: 7 - protein, 18 aa, Artificial Sequence
  Synthetic
EQRTESIIHRALYYDLIS

SEQ ID NO: 8 - protein, 29 aa, Artificial Sequence
  Synthetic
SLGAEHRTESVIHRALYYDLITNPDIHST

SEQ ID NO: 9 - protein, 20 aa, Artificial Sequence
  Synthetic
SLGAEHRTESVIHRALYYDL